European Patent Application EP 4 393 954 A1, published July 3, 2024. Title: ANTI-TNFR2 MONOCLONAL ANTIBODY AND APPLICATION THEREOF. Applicant: SHANGHAI CELGEN BIO-PHARMACEUTICAL CO., LTD. The sequence listing filed with the application follows.

SEQUENCE LISTING (107 sequences)

SEQ ID NO: 1 - protein, 115 aa, synthetic construct
  REGION 1..115: note = full length sequence of mouse mAb 16D2 VH
EVQLQQSEPELVKPGASVKIPCKASGYTFTDYNMDWVKQSHGKSLEWIGDINPNNGVTIYNQKFKGKATLTVDKSSSTAYMELRSLTSEDTAVYYCVILEYFDYWGQGTTLTVSS

SEQ ID NO: 2 - protein, 5 aa, synthetic construct
  REGION 1..5: note = mouse mAb 16D2 VHCDR1
DYNMD

SEQ ID NO: 3 - protein, 17 aa, synthetic construct
  REGION 1..17: note = mouse mAb 16D2 VHCDR2
DINPNNGVTIYNQKFKG

SEQ ID NO: 4 - protein, 6 aa, synthetic construct
  REGION 1..6: note = mouse mAb 16D2 VHCDR3
LEYFDY

SEQ ID NO: 5 - protein, 107 aa, synthetic construct
  REGION 1..107: note = full length sequence of mouse mAb 16D2 VL
DIVMTQSTSSMSVSLGDTVSITCHASQGISSNIGWLQQKPGKSFKGLIYHGTKLEDGVPSRFSGSGSGADYSLTISSLESEDFADYYCVQYAQFPRTFGGGTKLEIK

SEQ ID NO: 6 - protein, 11 aa, synthetic construct
  REGION 1..11: note = mouse mAb 16D2 VLCDR1
HASQGISSNIG

SEQ ID NO: 7 - protein, 7 aa, synthetic construct
  REGION 1..7: note = mouse mAb 16D2 VLCDR2
HGTKLED

SEQ ID NO: 8 - protein, 9 aa, synthetic construct
  REGION 1..9: note = mouse mAb 16D2 VLCDR3
VQYAQFPRT

SEQ ID NO: 9 - protein, 121 aa, synthetic construct
  REGION 1..121: note = full length sequence of mouse mAb 27F6 VH
EVQLQQSGTVLARPGASVKMSCKTSGYTFTSYWMHWVKQRPGQGLEWIGTIYPGNSDTSYNQKFKGKAKLTAVTSASTAYMELNSLTNEDSAVFYCTRENLLLRSYFFDYWGQGTTLTVSS

SEQ ID NO: 10 - protein, 5 aa, synthetic construct
  REGION 1..5: note = mouse mAb 27F6 VHCDR1
SYWMH

SEQ ID NO: 11 - protein, 17 aa, synthetic construct
  REGION 1..17: note = mouse mAb 27F6 VHCDR2
TIYPGNSDTSYNQKFKG

SEQ ID NO: 12 - protein, 12 aa, synthetic construct
  REGION 1..12: note = mouse mAb 27F6 VHCDR3
ENLLLRSYFFDY

SEQ ID NO: 13 - protein, 111 aa, synthetic construct
  REGION 1..111: note = full length sequence of mouse mAb 27F6 VL
DIVMTQSPASLAVSLGQRATISCKASQSVDYDGDSYLNWYQQKPGQPPKLLIYAASNLPSGIPARFSGSGSGTDFTLNIHPVEEEDAATYYCQQSNEDPRTFGGGTKLEIK

SEQ ID NO: 14 - protein, 15 aa, synthetic construct
  REGION 1..15: note = mouse mAb 27F6 VLCDR1
KASQSVDYDGDSYLN

SEQ ID NO: 15 - protein, 7 aa, synthetic construct
  REGION 1..7: note = mouse mAb 27F6 VLCDR2
AASNLPS

SEQ ID NO: 16 - protein, 9 aa, synthetic construct
  REGION 1..9: note = mouse mAb 27F6 VLCDR3
QQSNEDPRT

SEQ ID NO: 17 - protein, 123 aa, synthetic construct
  REGION 1..123: note = full length sequence of mouse mAb 29A1 VH
QVQLQQSGAEVVRPGASVTLSCKASGYTFSDYEMHWVKQTPVHGLEWIGAIDPETGDTAYNQKFKDKARVTADKSSSTAYMELRSLTSEDSAVYYCTRDIHYYGSSLSYFDYWGQGTTLTVSS

SEQ ID NO: 18 - protein, 5 aa, synthetic construct
  REGION 1..5: note = mouse mAb 29A1 VHCDR1
DYEMH

SEQ ID NO: 19 - protein, 17 aa, synthetic construct
  REGION 1..17: note = mouse mAb 29A1 VHCDR2
AIDPETGDTAYNQKFKD

SEQ ID NO: 20 - protein, 14 aa, synthetic construct
  REGION 1..14: note = mouse mAb 29A1 VHCDR3
DIHYYGSSLSYFDY

SEQ ID NO: 21 - protein, 107 aa, synthetic construct
  REGION 1..107: note = full length sequence of mouse mAb 29A1 VL
DIVMTQSQKFMSTSVGDRVSVTCKASQNVGTNVAWYQQKPGQSPKVMIYSASYRYSGAPDRFTGSGSGTDFTLTVNNVQSEDLAEYFCQQYKTYPYTFGGGTKLEIE

SEQ ID NO: 22 - protein, 11 aa, synthetic construct
  REGION 1..11: note = mouse mAb 29A1 VLCDR1
KASQNVGTNVA

SEQ ID NO: 23 - protein, 7 aa, synthetic construct
  REGION 1..7: note = mouse mAb 29A1 VLCDR2
SASYRYS

SEQ ID NO: 24 - protein, 9 aa, synthetic construct
  REGION 1..9: note = mouse mAb 29A1 VLCDR3
QQYKTYPYT

SEQ ID NO: 25 - protein, 119 aa, synthetic construct
  REGION 1..119: note = full length sequence of mouse mAb 7F2 VH
QVTLKESGPGILQPSQTLSLTCSFSGFSLNTFGLGVGWIRQPSGKGLEWLTHIWWNDDKYYNPALKSRLTISRDTSENLVFLKIANVDTADTATYYCARIEGLRRFDYWGQGTTLTVSS

SEQ ID NO: 26 - protein, 7 aa, synthetic construct
  REGION 1..7: note = mouse mAb 7F2 VHCDR1
TFGLGVG

SEQ ID NO: 27 - protein, 16 aa, synthetic construct
  REGION 1..16: note = mouse mAb 7F2 VHCDR2
HIWWNDDKYYNPALKS

SEQ ID NO: 28 - protein, 9 aa, synthetic construct
  REGION 1..9: note = mouse mAb 7F2 VHCDR3
IEGLRRFDY

SEQ ID NO: 29 - protein, 106 aa, synthetic construct
  REGION 1..106: note = full length sequence of mouse mAb 7F2 VL
DIQMTQSPSSLSASLGGKVTITCKTSQDINKFIAWYQHKPGKGPRLLIHYTSTLQPGIPSRFSGSGSGRDYSFSISDLEPEDIATYYCLQYANLWAFGGGTKLEIK

SEQ ID NO: 30 - protein, 11 aa, synthetic construct
  REGION 1..11: note = mouse mAb 7F2 VLCDR1
KTSQDINKFIA

SEQ ID NO: 31 - protein, 7 aa, synthetic construct
  REGION 1..7: note = mouse mAb 7F2 VLCDR2
YTSTLQP

SEQ ID NO: 32 - protein, 8 aa, synthetic construct
  REGION 1..8: note = mouse mAb 7F2 VLCDR3
LQYANLWA

SEQ ID NO: 33 - protein, 119 aa, synthetic construct
  REGION 1..119: note = full length sequence of mouse mAb 11G2 VH
QVHLQQSGPELVKPGAPVKLSCKASGYTFITYDINWVKQRPGQGLEWIGWIYPRDGNTQFNENFKGKATMSVDESSSTAYMEVHSLTSEDSAVYFCARGDRDYGYFDVWGTGTTVSVSS

SEQ ID NO: 34 - protein, 5 aa, synthetic construct
  REGION 1..5: note = mouse mAb 11G2 VHCDR1
TYDIN

SEQ ID NO: 35 - protein, 17 aa, synthetic construct
  REGION 1..17: note = mouse mAb 11G2 VHCDR2
WIYPRDGNTQFNENFKG

SEQ ID NO: 36 - protein, 10 aa, synthetic construct
  REGION 1..10: note = mouse mAb 11G2 VHCDR3
GDRDYGYFDV

SEQ ID NO: 37 - protein, 107 aa, synthetic construct
  REGION 1..107: note = full length sequence of mouse mAb 11G2 VL
DIQMTPTTSSLSVSLGDRVTISYRASQDISNYLNWYQQKPDGTVKLLIYFKSKLHSGVPSRFSGSGSGTDFSLTIANLEQEDIATYFCQQGNTLPLTFGVGTRLALK

SEQ ID NO: 38 - protein, 11 aa, synthetic construct
  REGION 1..11: note = mouse mAb 11G2 VLCDR1
RASQDISNYLN

SEQ ID NO: 39 - protein, 7 aa, synthetic construct
  REGION 1..7: note = mouse mAb 11G2 VLCDR2
FKSKLHS

SEQ ID NO: 40 - protein, 9 aa, synthetic construct
  REGION 1..9: note = mouse mAb 11G2 VLCDR3
QQGNTLPLT

SEQ ID NO: 41 - protein, 118 aa, synthetic construct
  REGION 1..118: note = full length sequence of mouse mAb 12E12 VH
EVQLQQSGAELVKPGASVKLSCTVSGFNIKDFYIHWVKQRPEQGLEWIGRVDPEDGNTEYAPNFQDRATMTTDTSSNTAYLQLSSLTSVDTAVYYCSTWDGFSYFDYWGLGTTLTVSS

SEQ ID NO: 42 - protein, 5 aa, synthetic construct
  REGION 1..5: note = mouse mAb 12E12 VHCDR1
DFYIH

SEQ ID NO: 43 - protein, 17 aa, synthetic construct
  REGION 1..17: note = mouse mAb 12E12 VHCDR2
RVDPEDGNTEYAPNFQD

SEQ ID NO: 44 - protein, 9 aa, synthetic construct
  REGION 1..9: note = mouse mAb 12E12 VHCDR3
WDGFSYFDY

SEQ ID NO: 45 - protein, 109 aa, synthetic construct
  REGION 1..109: note = full length sequence of mouse mAb 12E12 VL
QAVVTQESALTTSPGETVTLTCRSSTGPVTTNNYANWVQEKPDHLFTGLIGGTNDRAPGVPARFSGSLIGDKTALTITGTQTEDEAVYFCALWYRNHWVFGGGTKLTVL

SEQ ID NO: 46 - protein, 14 aa, synthetic construct
  REGION 1..14: note = mouse mAb 12E12 VLCDR1
RSSTGPVTTNNYAN

SEQ ID NO: 47 - protein, 7 aa, synthetic construct
  REGION 1..7: note = mouse mAb 12E12 VLCDR2
GTNDRAP

SEQ ID NO: 48 - protein, 9 aa, synthetic construct
  REGION 1..9: note = mouse mAb 12E12 VLCDR3
ALWYRNHWV

SEQ ID NO: 49 - protein, 122 aa, synthetic construct
  REGION 1..122: note = full length sequence of mouse mAb 13F5 VH
QVQLQQSGAELVRPGTSVKMSCKASGYTFTNYWIGWTKQRPGHGLEWIGDIFPGGDFTNYNEKFKGKATLTADKSSSTAYLQFSSLTSEDSAIYYCSRRRFTTIVAPGFDYWGQGTTLTVSS

SEQ ID NO: 50 - protein, 5 aa, synthetic construct
  REGION 1..5: note = mouse mAb 13F5 VHCDR1
NYWIG

SEQ ID NO: 51 - protein, 17 aa, synthetic construct
  REGION 1..17: note = mouse mAb 13F5 VHCDR2
DIFPGGDFTNYNEKFKG

SEQ ID NO: 52 - protein, 13 aa, synthetic construct
  REGION 1..13: note = mouse mAb 13F5 VHCDR3
RRFTTIVAPGFDY

SEQ ID NO: 53 - protein, 115 aa, synthetic construct
  REGION 1..115: note = full length sequence of mouse mAb 13F5 VL
QLVLTQSSSASFSLGASAKLTCTLSSQHSMYTIEWYQQQPLKPPKFVMELKKDGSHSTGDGIPDRFSGSSSGADRYLNISNIQPEDEAIYICGVGDTIKEQFVYVFGGGTEVTVL

SEQ ID NO: 54 - protein, 12 aa, synthetic construct
  REGION 1..12: note = mouse mAb 13F5 VLCDR1
TLSSQHSMYTIE

SEQ ID NO: 55 - protein, 7 aa, synthetic construct
  REGION 1..7: note = mouse mAb 13F5 VLCDR2
GSHSTGD

SEQ ID NO: 56 - protein, 13 aa, synthetic construct
  REGION 1..13: note = mouse mAb 13F5 VLCDR3
GVGDTIKEQFVYV

SEQ ID NO: 57 - protein, 114 aa, synthetic construct
  REGION 1..114: note = full length sequence of mouse mAb 18A2 VH
DVQLQESGPGLVKPSQSLSLTCSVTGYSITSGYYWNWIRQFPGNKLEWMGYISYDGSNNYNPSLKKRISITRDTSKNQFFLKLNSVTTEDTATYYCTGGSGTSWGQGTLVTVSA

SEQ ID NO: 58 - protein, 6 aa, synthetic construct
  REGION 1..6: note = mouse mAb 18A2 VHCDR1
SGYYWN

SEQ ID NO: 59 - protein, 16 aa, synthetic construct
  REGION 1..16: note = mouse mAb 18A2 VHCDR2
YISYDGSNNYNPSLKK

SEQ ID NO: 60 - protein, 5 aa, synthetic construct
  REGION 1..5: note = mouse mAb 18A2 VHCDR3
GSGTS

SEQ ID NO: 61 - protein, 107 aa, synthetic construct
  REGION 1..107: note = full length sequence of mouse mAb 18A2 VL
DIVMTQSHKFMSTSVGDRVSITCKASQDVTTGIAWYQQKPGQSPKLLIYSASNRFTGVPDRFTGSGSGTDFTFTISSVQAEDLAVYFCQQHYSTPFTFGSGTKLEIQ

SEQ ID NO: 62 - protein, 11 aa, synthetic construct
  REGION 1..11: note = mouse mAb 18A2 VLCDR1
KASQDVTTGIA

SEQ ID NO: 63 - protein, 7 aa, synthetic construct
  REGION 1..7: note = mouse mAb 18A2 VLCDR2
SASNRFT

SEQ ID NO: 64 - protein, 9 aa, synthetic construct
  REGION 1..9: note = mouse mAb 18A2 VLCDR3
QQHYSTPFT

SEQ ID NO: 65 - protein, 120 aa, synthetic construct
  REGION 1..120: note = full length sequence of mouse mAb 33C12 VH
DVKLVESGGGLVKPGGSLKLSCAASGFTFSDYTMSWVRQTPEKRLEWVATISTGGSYTYYPDSVKGRFTISRDNAKNTLYLQMSSLKSEDTAMYYCTRDGGYDGDYFDYWGQGTTLTVSS

SEQ ID NO: 66 - protein, 5 aa, synthetic construct
  REGION 1..5: note = mouse mAb 33C12 VHCDR1
DYTMS

SEQ ID NO: 67 - protein, 17 aa, synthetic construct
  REGION 1..17: note = mouse mAb 33C12 VHCDR2
TISTGGSYTYYPDSVKG

SEQ ID NO: 68 - protein, 11 aa, synthetic construct
  REGION 1..11: note = mouse mAb 33C12 VHCDR3
DGGYDGDYFDY

SEQ ID NO: 69 - protein, 108 aa, synthetic construct
  REGION 1..108: note = full length sequence of mouse mAb 33C12 VL
ENVLTQSPAIMSASPGEKVTMTCRASSSVSSSYLHWYQQKSGASPKLWIYRTSNLASGVPARFSGSGSGTSYSLTISSVEAEDAATYYCQQYSGYPLTFGAGTRLELK

SEQ ID NO: 70 - protein, 12 aa, synthetic construct
  REGION 1..12: note = mouse mAb 33C12 VLCDR1
RASSSVSSSYLH

SEQ ID NO: 71 - protein, 7 aa, synthetic construct
  REGION 1..7: note = mouse mAb 33C12 VLCDR2
RTSNLAS

SEQ ID NO: 72 - protein, 9 aa, synthetic construct
  REGION 1..9: note = mouse mAb 33C12 VLCDR3
QQYSGYPLT

SEQ ID NO: 73 - protein, 119 aa, synthetic construct
  REGION 1..119: note = full length sequence of humanized Ab 11G2-huVH1
QVQLVQSGAEVKKPGASVKLSCKASGYTFITYDINWVRQAPGQGLEWIGWIYPRDGNTQFNENFKGKATMTVDESTSTAYMEVRSLRSDDTAVYYCARGDRDYGYFDVWGQGTTVTVSS

SEQ ID NO: 74 - protein, 119 aa, synthetic construct
  REGION 1..119: note = full length sequence of humanized Ab 11G2-huVH2
QVQLVQSGAEVKKPGASVKVSCKASGYTFITYDINWVRQAPGQGLEWIGWIYPRDGNTQFNENFKGRVTMTTDTSTSTAYMELRSLRSDDTAVYYCARGDRDYGYFDVWGQGTTVTVSS

SEQ ID NO: 75 - protein, 119 aa, synthetic construct
  REGION 1..119: note = full length sequence of humanized Ab 11G2-huVH3
QVQLVQSGAEVKKPGASVKVSCKASGYTFITYDINWVRQATGQGLEWIGWIYPRDGNTQFNENFQGRVTMTRNTSISTAYMELSSLRSEDTAVYYCARGDRDYGYFDVWGQGTTVTVSS

SEQ ID NO: 76 - protein, 119 aa, synthetic construct
  REGION 1..119: note = full length sequence of humanized Ab 11G2-huVH4
QVQLVQSGAEVKKPGASVKVSCKASGYTFITYDINWVRQAPGQGLEWIGWIYPRDGNTQYAQKFQGRVTMTTDTSTSTAYMELRSLRSDDTAVYYCARGDRDYGYFDVWGQGTTVTVSS

SEQ ID NO: 77 - protein, 119 aa, synthetic construct
  REGION 1..119: note = full length sequence of humanized Ab 11G2-huVH5
QVQLVQSGAEVKKPGASVKVSCKASGYTFITYDINWVRQATGQGLEWIGWIYPRDGNTQYAQKFQGRVTMTRNTSISTAYMELSSLRSEDTAVYYCARGDRDYGYFDVWGQGTTVTVSS

SEQ ID NO: 78 - protein, 107 aa, synthetic construct
  REGION 1..107: note = full length sequence of humanized Ab 11G2-huVL1
DIQMTPSTSSLSASVGDRVTITCRASQDISNYLNWYQQKPGKAVKLLIYFKSKLHSGVPSRFSGSGSGTDFTLTISSLQPEDFATYYCQQGNTLPLTFGGGTKLELK

SEQ ID NO: 79 - protein, 107 aa, synthetic construct
  REGION 1..107: note = full length sequence of humanized Ab 11G2-huVL2
DIQMTQSPSSLSASVGDRVTITCRASQDISNYLNWYQQKPGKAPKLLIYFKSKLHSGVPSRFSGSGSGTDFTLTISSLQPEDFATYYCQQGNTLPLTFGGGTKLEIK

SEQ ID NO: 80 - protein, 107 aa, synthetic construct
  REGION 1..107: note = full length sequence of humanized Ab 11G2-huVL3
DIQMTQSPSSLSASVGDRVTITCQASQDISNYLNWYQQKPGKAPKLLIYFKSKLETGVPSRFSGSGSGTDFTFTISSLQPEDIATYYCQQGNTLPLTFGGGTKLEIK

SEQ ID NO: 81 - protein, 120 aa, synthetic construct
  REGION 1..120: note = full length sequence of humanized Ab 33C12-huVH1
DVQLVESGGGLVKPGGSLRLSCAASGFTFSDYTMSWVRQAPGKGLEWVATISTGGSYTYYPDSVKGRFTISRDNAKNTLYLQMSSLRAEDTAVYYCTRDGGYDGDYFDYWGQGTTVTVSS

SEQ ID NO: 82 - protein, 120 aa, synthetic construct
  REGION 1..120: note = full length sequence of humanized Ab 33C12-huVH2
EVQLVESGGGLVKPGGSLRLSCAASGFTFSDYTMSWVRQAPGKGLEWVATISTGGSYTYYPDSVKGRFTISRDNAKNTLYLQMSSLRAEDTAVYYCARDGGYDGDYFDYWGQGTTVTVSS

SEQ ID NO: 83 - protein, 120 aa, synthetic construct
  REGION 1..120: note = full length sequence of humanized Ab 33C12-huVH3
EVQLVESGGGLVKPGGSLRLSCAASGFTFSDYTMSWVRQAPGKGLEWVATISTGGSYTYYADSVKGRFTISRDNAKNSLYLQMNSLRAEDTAVYYCARDGGYDGDYFDYWGQGTTVTVSS

SEQ ID NO: 84 - protein, 108 aa, synthetic construct
  REGION 1..108: note = full length sequence of humanized Ab 33C12-huVL1
ENVLTQSPATLSLSPGERATMSCRASSSVSSSYLHWYQQKPGQAPRLWIYRTSNLASGVPARFSGSGSGTDYTLTISRVEPEDFAVYYCQQYSGYPLTFGGGTKLEIK

SEQ ID NO: 85 - protein, 108 aa, synthetic construct
  REGION 1..108: note = full length sequence of humanized Ab 33C12-huVL2
ENVLTQSPATLSLSPGERATLSCRASSSVSSSYLHWYQQKPGQAPRLWIYRTSNLASGVPARFSGSGSGTDFTLTISRLEPEDFAVYYCQQYSGYPLTFGGGTKLEIK

SEQ ID NO: 86 - protein, 108 aa, synthetic construct
  REGION 1..108: note = full length sequence of humanized Ab 33C12-huVL3
EIVLTQSPATLSLSPGERATLSCRASSSVSSSYLHWYQQKPGQAPRLLIYRTSNLATGIPDRFSGSGSGTDFTLTISRLEPEDFAVYYCQQYSGYPLTFGGGTKLEIK

SEQ ID NO: 87 - protein, 18 aa, synthetic construct
  REGION 1..18: note = CDR2 of humanized Ab 11G2-huVH3
WIYPRDGNTQFNENFQGR

SEQ ID NO: 88 - protein, 18 aa, synthetic construct
  REGION 1..18: note = CDR2 of humanized Ab 11G2-huVH4/VH5
WIYPRDGNTQYAQKFQGR

SEQ ID NO: 89 - protein, 7 aa, synthetic construct
  REGION 1..7: note = CDR2 of humanized Ab 11G2-huVL3
FKSKLET

SEQ ID NO: 90 - protein, 17 aa, synthetic construct
  REGION 1..17: note = CDR2 of humanized Ab 33C12-huVH3
TISTGGSYTYYADSVKG

SEQ ID NO: 91 - protein, 7 aa, synthetic construct
  REGION 1..7: note = CDR2 of humanized Ab 33C12-huVL3
RTSNLAT

SEQ ID NO: 92 - protein, 118 aa, synthetic construct
  REGION 1..118: note = full length sequence of humanized Ab 12E12-huVH1
EVQLVQSGAEVKKPGASVKLSCTVSGFNIKDFYIHWVRQAPGQGLEWIGRVDPEDGNTEYAPNFQDRATMTTDTSTNTAYLELSSLRSEDTAVYYCSTWDGFSYFDYWGQGTTVTVSS

SEQ ID NO: 93 - protein, 118 aa, synthetic construct
  REGION 1..118: note = full length sequence of humanized Ab 12E12-huVH2
QVQLVQSGAEVKKPGASVKVSCKVSGFNIKDFYIHWVRQAPGQGLEWIGRVDPEDGNTEYAPNFQDRATMTTDTSTSTAYLELSSLRSEDTAVYYCSTWDGFSYFDYWGQGTTVTVSS

SEQ ID NO: 94 - protein, 118 aa, synthetic construct
  REGION 1..118: note = full length sequence of humanized Ab 12E12-huVH3
QVQLVQSGAEVKKPGASVKVSCKVSGFNIKDFYIHWVRQAPGKGLEWMGRVDPEDGNTEYAQKFQGRVTMTTDTSTDTAYMELSSLRSEDTAVYYCSTWDGFSYFDYWGQGTTVTVSS

SEQ ID NO: 95 - protein, 17 aa, synthetic construct
  REGION 1..17: note = CDR2 of humanized Ab 12E12-huVH3
RVDPEDGNTEYAQKFQG

SEQ ID NO: 96 - protein, 118 aa, synthetic construct
  REGION 1..118: note = full length sequence of humanized Ab 12E12-huVH4
EVQLVQSGAEVKKPGATVKISCKVSGFNIKDFYIHWVQQAPGKGLEWIGRVDPEDGNTEYAPNFQDRVTITADTSTDTAYMELSSLRSEDTAVYYCSTWDGFSYFDYWGQGTTVTVSS

SEQ ID NO: 97 - protein, 118 aa, synthetic construct
  REGION 1..118: note = full length sequence of humanized Ab 12E12-huVH5
EVQLVQSGAEVKKPGATVKISCKVSGFNIKDFYIHWVQQAPGKGLEWIGRVDPEDGNTEYAEKFQGRVTITADTSTDTAYMELSSLRSEDTAVYYCSTWDGFSYFDYWGQGTTVTVSS

SEQ ID NO: 98 - protein, 17 aa, synthetic construct
  REGION 1..17: note = CDR2 of humanized Ab 12E12-huVH5
RVDPEDGNTEYAEKFQG

SEQ ID NO: 99 - protein, 118 aa, synthetic construct
  REGION 1..118: note = full length sequence of humanized Ab 12E12-huVH6
QVQLVQSGAEVKKPGASVKVSCKASGYTITDFYIHWVRQAPGQGLEWIGRVDPEDGNTEYAPNFQDRATMTTDTSTSTAYLELSSLRSEDTAVYYCSTWDGFSYFDYWGQGTTVTVSS

SEQ ID NO: 100 - protein, 118 aa, synthetic construct
  REGION 1..118: note = full length sequence of humanized Ab 12E12-huVH7
QVQLVQSGAEVKKPGASVKVSCKASGYTITDFYIHWVRQAPGKGLEWMGRVDPEDGNTEYAQKFQGRVTMTTDTSTDTAYMELSSLRSEDTAVYYCSTWDGFSYFDYWGQGTTVTVSS

SEQ ID NO: 101 - protein, 118 aa, synthetic construct
  REGION 1..118: note = full length sequence of humanized Ab 12E12-huVH8
EVQLVQSGAEVKKPGATVKISCKVSGYTITDFYIHWVQQAPGKGLEWMGRVDPEDGNTEYAPNFQDRVTITADTSTDTAYMELSSLRSEDTAVYYCSTWDGFSYFDYWGQGTTVTVSS

SEQ ID NO: 102 - protein, 109 aa, synthetic construct
  REGION 1..109: note = full length sequence of humanized Ab 12E12-huVL1
QAVVTQEPSLTVSPGGTVTLTCRSSTGPVTTNNYANWVQQKPGQAFRGLIGGTNDRAPGVPARFSGSLIGDKTALTLSGVQPEDEAEYYCALWYRNHWVFGGGTKLTVL

SEQ ID NO: 103 - protein, 109 aa, synthetic construct
  REGION 1..109: note = full length sequence of humanized Ab 12E12-huVL2
QAVVTQEPSLTVSPGGTVTLTCRSSTGPVTTNNYANWVQQKPGQAFRGLIGGTNDRAPGVPARFSGSLLGGKAALTLSGAQPEDEAEYYCALWYRNHWVFGGGTKLTVL

SEQ ID NO: 104 - protein, 109 aa, synthetic construct
  REGION 1..109: note = full length sequence of humanized Ab 12E12-huVL3
QAVVTQEPSLTVSPGGTVTLTCRSSTGPVTTNNYANWFQQKPGQAPRTLIGGTNDRAPGVPARFSGSLLGGKAALTLSGAQPEDEAEYYCALWYRNHWVFGGGTKLTVL

SEQ ID NO: 105 - protein, 110 aa, synthetic construct
  REGION 1..110: note = full length sequence of humanized Ab 12E12-huVL4
EAVVTQSPATLSLSPGERATLSCRSSTGPVTTNNYANWVQQKPGQAFRGLIGGTNDRAPGIPARFSGSGSGTDTTLTISSLQPEDFAVYYCALWYRNHWVFGGGTKLEIK

SEQ ID NO: 106 - protein, 110 aa, synthetic construct
  REGION 1..110: note = full length sequence of humanized Ab 12E12-huVL5
EIVMTQSPATLSLSPGERATLSCRSSTGPVTTNNYANWYQQKPGQAPRLLIGGTNDRATGIPARFSGSGSGTDTTLTISSLQPEDFAVYYCALWYRNHWVFGGGTKLEIK

SEQ ID NO: 107 - protein, 7 aa, synthetic construct
  REGION 1..7: note = CDR2 of humanized Ab 12E12-huVL5
GTNDRAT